European Patent Application EP 4 585 688 A1, published July 16, 2025. Title: Nucleic Acid Molecules, Fusion Proteins, and mRNA Vaccines with Enhanced Antigen Presentation by Recruiting Ligands. Applicant: WESTGENE BIOPHARMA CO., LTD. The sequence listing filed with the application follows.

SEQUENCE LISTING (21 sequences)

SEQ ID NO: 1 - skipped

SEQ ID NO: 2 - DNA, 15 bp, synthetic construct
  source 1..15: mol_type = other DNA
ggggsggggsggggs

SEQ ID NO: 3 - DNA, 30 bp, synthetic construct
  source 1..30: mol_type = other DNA
ggggsggggsggggsggggsggggsggggs

SEQ ID NO: 4 - DNA, 30 bp, synthetic construct
  source 1..30: mol_type = other DNA
ggsggsggsggsggsggsggsggsggsggs

SEQ ID NO: 5 - DNA, 30 bp, synthetic construct
  source 1..30: mol_type = other DNA
gsggsggsggsggsggsggsggsggsggsg

SEQ ID NO: 6-17 - skipped (12 entries)

SEQ ID NO: 18 - DNA, 72 bp, synthetic construct
  source 1..72: mol_type = other DNA
aggcaaaaatcaaaatcaatcatcatcacaacatcaacaatcaatcatcaacacatcatcaagacagccacc

SEQ ID NO: 19 - DNA, 280 bp, synthetic construct
  source 1..280: mol_type = other DNA
tgatgagctcgctttcttgctgtccaatttctattaaaggttcctttgttccctaagtccaactactaaactgggggatattatgaagggccttgagcatctggattctgcctaataaaaaacatttattttcattgctgcgtcgagagctcgctttcttgctgtccaatttctattaaaggttcctttgttccctaagtccaactactaaactgggggatattatgaagggccttgagcatctggattctgcctaataaaaaacatttattttcattgc

SEQ ID NO: 20 - DNA, 106 bp, synthetic construct
  source 1..106: mol_type = other DNA
aaaaaaaaaaaaaaaaaaaaaaaaaaaaaaaaaaaaaaaaaaaaaaaaaagtcttcaaaaaaaaaaaaaaaaaaaaaaaaaaaaaaaaaaaaaaaaaaaaaaaaaa

SEQ ID NO: 21 - skipped